European Patent Application EP 4 265 735 A1, published October 25, 2023. Title: PCR-Multiplexing durch Zielsequenz-Unabhängige-Reportermoleküle mit unterscheidbaren Signalstäken. Applicant: Hahn-Schickard-Gesellschaft. Application EP. The sequence listing filed with the application follows.

SEQUENCE LISTING (22 sequences)

SEQ ID NO: 1 - DNA, 18 bp, synthetic construct
  source 1..18: mol_type = other DNA
ggcctgctgaaaatgact

SEQ ID NO: 2 - DNA, 25 bp, synthetic construct
  source 1..25: mol_type = other DNA
acaaaatgattctgaattagctgta

SEQ ID NO: 3 - DNA, 21 bp, synthetic construct
  source 1..21: mol_type = other DNA
gacccactccatcgagatttc

SEQ ID NO: 4 - DNA, 23 bp, synthetic construct
  source 1..23: mol_type = other DNA
gcttgctctgataggaaaatgag

SEQ ID NO: 5 - DNA, 43 bp, synthetic construct
  source 1..43: mol_type = other DNA
ctccagttcggtccagctccaactaccacaagtttatattcag

SEQ ID NO: 6 - DNA, 39 bp, synthetic construct
  source 1..39: mol_type = other DNA
gatacagggtccactggcgtaggcaagagtgccttgacg

SEQ ID NO: 7 - DNA, 41 bp, synthetic construct
  source 1..41: mol_type = other DNA
atgtcccaggtgcatggcgtaggcaagagtgccttgacgat

SEQ ID NO: 8 - DNA, 40 bp, synthetic construct
  source 1..40: mol_type = other DNA
aggtaggctcacttggcgtaggcaagagtgccttgacgat

SEQ ID NO: 9 - DNA, 54 bp, synthetic construct
  source 1..54: mol_type = other DNA
acatgctcatgttgtgtctgtagctagaccaaaatcacctatttttactgtgag

SEQ ID NO: 10 - DNA, 54 bp, synthetic construct
  source 1..54: mol_type = other DNA
gtgttcctcacatgctactgtagctagaccaaaatcacctatttttactgtgag

SEQ ID NO: 11 - DNA, 45 bp, synthetic construct
  source 1..45: mol_type = other DNA
  modified_base 1: mod_base = OTHER; note = BMN-Q1
  modified_base 22: mod_base = OTHER; note = DY-530
gaccggccaagacgcgccggtctgttcactgaccgaactggagca

SEQ ID NO: 12 - DNA, 45 bp, synthetic construct
  source 1..45: mol_type = other DNA
  modified_base 1: mod_base = OTHER; note = BHQ-1
  modified_base 22: mod_base = OTHER; note = BMN-536
gaccgcactagtagatgcggtctgtcgtggaccctgtatcgagca

SEQ ID NO: 13 - DNA, 46 bp, synthetic construct
  source 1..46: mol_type = other DNA
  modified_base 1: mod_base = OTHER; note = BHQ-2
  modified_base 22: mod_base = OTHER; note = Cy5
gaccggctaagacgcgccggtctgttgcacctgggacatcgactat

SEQ ID NO: 14 - DNA, 46 bp, synthetic construct
  source 1..46: mol_type = other DNA
  modified_base 1: mod_base = OTHER; note = BHQ-2
  modified_base 22: mod_base = OTHER; note = Atto-647N
gacgcgtagtacagaacgcgtctgttcagtgagcctacctgccttc

SEQ ID NO: 15 - DNA, 47 bp, synthetic construct
  source 1..47: mol_type = other DNA
  modified_base 1: mod_base = OTHER; note = BHQ-1
  modified_base 20: mod_base = OTHER; note = FAM
atgccgattagatgcggcattcgatcacacaacatgagcatgtgtac

SEQ ID NO: 16 - DNA, 45 bp, synthetic construct
  source 1..45: mol_type = other DNA
  modified_base 1: mod_base = OTHER; note = BMN-Q1
  modified_base 20: mod_base = OTHER; note = Atto-488
atccgccaagacgcgcggattagcatgtgaggaacacgatgacac

SEQ ID NO: 17 - DNA, 160 bp, unidentified
  source 1..160: mol_type = other DNA
caaactgatgggacccactccatcgagatttcactgtagctagaccaaaatcacctatttttactgtgaggtcttcatgaagaaatatatctgaggtgtagtaagtaaaggaaaacagtagatctcattttcctatcagagcaagcattatgaagagttt

SEQ ID NO: 18 - DNA, 160 bp, unidentified
  source 1..160: mol_type = other DNA
caaactgatgggacccactccatcgagatttctctgtagctagaccaaaatcacctatttttactgtgaggtcttcatgaagaaatatatctgaggtgtagtaagtaaaggaaaacagtagatctcattttcctatcagagcaagcattatgaagagttt

SEQ ID NO: 19 - DNA, 131 bp, unidentified
  source 1..131: mol_type = other DNA
cattttcattatttttattataaggcctgctgaaaatgactgaatataaacttgtggtagttggagctggtggcgtaggcaagagtgccttgacgatacagctaattcagaatcattttgtggacgaatat

SEQ ID NO: 20 - DNA, 131 bp, unidentified
  source 1..131: mol_type = other DNA
cattttcattatttttattataaggcctgctgaaaatgactgaatataaacttgtggtagttggagctgctggcgtaggcaagagtgccttgacgatacagctaattcagaatcattttgtggacgaatat

SEQ ID NO: 21 - DNA, 131 bp, unidentified
  source 1..131: mol_type = other DNA
cattttcattatttttattataaggcctgctgaaaatgactgaatataaacttgtggtagttggagctgatggcgtaggcaagagtgccttgacgatacagctaattcagaatcattttgtggacgaatat

SEQ ID NO: 22 - DNA, 131 bp, unidentified
  source 1..131: mol_type = other DNA
cattttcattatttttattataaggcctgctgaaaatgactgaatataaacttgtggtagttggagctgttggcgtaggcaagagtgccttgacgatacagctaattcagaatcattttgtggacgaatat